European Patent Application EP 4 696 773 A1, published February 18, 2026. Title: SARNA DELIVERY SYSTEM, PREPARATION METHOD THEREFOR AND USE THEREOF. Applicant: Zhejiang Free Trade Zone Hongan Base Biotechnology Co., Ltd. Application WO. The sequence listing filed with the application follows.

SEQUENCE LISTING (15 sequences)

SEQ ID NO: 1 - DNA, 12361 bp, synthetic construct
  source 1..12361: mol_type = other DNA
atgggcggcgcatgagagaagcccagaccaattacctacccaaaatggagaaagttcacgttgacatcgaggaagacagcccattcctcagagctttgcagcggagcttcccgcagtttgaggtagaagccaagcaggtcactgataatgaccatgctaatgccagagcgttttcgcatctggcttcaaaactgatcgaaacggaggtggacccatccgacacgatccttgacattggaagtgcgcccgcccgcagaatgtattctaagcacaagtatcattgtatctgtccgatgagatgtgcggaagatccggacagattgtataagtatgcaactaagctgaagaaaaactgtaaggaaataactgataaggaattggacaagaaaatgaaggagctcgccgccgtcatgagcgaccctgacctggaaactgagactatgtgcctccacgacgacgagtcgtgtcgctacgaagggcaagtcgctgtttaccaggatgtatacgcggttgacggaccgacaagtctctatcaccaagccaataagggagttagagtcgcctactggataggctttgacaccaccccttttatgtttaagaacttggctggagcatatccatcatactctaccaactgggccgacgaaaccgtgttaacggctcgtaacataggcctatgcagctctgacgttatggagcggtcacgtagagggatgtccattcttagaaagaagtatttgaaaccatccaacaatgttctattctctgttggctcgaccatctaccacgagaagagggacttactgaggagctggcacctgccgtctgtatttcacttacgtggcaagcaaaattacacatgtcggtgtgagactatagttagttgcgacgggtacgtcgttaaaagaatagctatcagtccaggcctgtatgggaagccttcaggctatgctgctacgatgcaccgcgagggattcttgtgctgcaaagtgacagacacattgaacggggagagggtctcttttcccgtgtgcacgtatgtgccagctacattgtgtgaccaaatgactggcatactggcaacagatgtcagtgcggacgacgcgcaaaaactgctggttgggctcaaccagcgtatagtcgtcaacggtcgcacccagagaaacaccaataccatgaaaaattaccttttgcccgtagtggcccaggcatttgctaggtgggcaaaggaatataaggaagatcaagaagatgaaaggccactaggactacgagatagacagttagtcatggggtgttgttgggcttttagaaggcacaagataacatctatttataagcgcccggatacccaaaccatcatcaaagtgaacagcgatttccactcattcgtgctgcccaggataggcagtaacacattggagatcgggctgagaacaagaatcaggaaaatgttagaggagcacaaggagccgtcacctctcattaccgccgaggacgtacaagaagctaagtgcgcagccgatgaggctaaggaggtgcgtgaagccgaggagttgcgcgcagctctaccacctttggcagctgatgttgaggagcccactctggaagccgatgtcgacttgatgttacaagaggctggggccggctcagtggagacacctcgtggcttgataaaggttaccagctacgctggcgaggacaagatcggctcttacgctgtgctttctccgcaggctgtactcaagagtgaaaaattatcttgcatccaccctctcgctgaacaagtcatagtgataacacactctggccgaaaagggcgttatgccgtggaaccataccatggtaaagtagtggtgccagagggacatgcaatacccgtccaggactttcaagctctgagtgaaagtgccaccattgtgtacaacgaacgtgagttcgtaaacaggtacctgcaccatattgccacacatggaggagcgctgaacactgatgaagaatattacaaaactgtcaagcccagcgagcacgacggcgaatacctgtacgacatcgacaggaaacagtgcgtcaagaaagaactagtcactgggctagggctcacaggcgagctggtggatcctcccttccatgaattcgcctacgagagtctgagaacacgaccagccgctccttaccaagtaccaaccataggggtgtatggcgtgccaggatcaggcaagtctggcatcattaaaagcgcagtcaccaaaaaagatctagtggtgagcgccaagaaagaaaactgtgcagaaattataagggacgtcaagaaaatgaaagggctggacgtcaatgccagaactgtggactcagtgctcttgaatggatgcaaacaccccgtagagaccctgtatattgacgaagcttttgcttgtcatgcaggtactctcagagcgctcatagccattataagacctaaaaaggcagtgctctgcggggatcccaaacagtgcggtttttttaacatgatgtgcctgaaagtgcattttaaccacgagatttgcacacaagtcttccacaaaagcatctctcgccgttgcactaaatctgtgacttcggtcgtctcaaccttgttttacgacaaaaaaatgagaacgacgaatccgaaagagactaagattgtgattgacactaccggcagtaccaaacctaagcaggacgatctcattctcacttgtttcagagggtgggtgaagcagttgcaaatagattacaaaggcaacgaaataatgacggcagctgcctctcaagggctgacccgtaaaggtgtgtatgccgttcggtacaaggtgaatgaaaatcctctgtacgcacccacctcagaacatgtgaacgtcctactgacccgcacggaggaccgcatcgtgtggaaaacactagccggcgacccatggataaaaacactgactgccaagtaccctgggaatttcactgccacgatagaggagtggcaagcagagcatgatgccatcatgaggcacatcttggagagaccggaccctaccgacgtcttccagaataaggcaaacgtgtgttgggccaaggctttagtgccggtgctgaagaccgctggcatagacatgaccactgaacaatggaacactgtggattattttgaaacggacaaagctcactcagcagagatagtattgaaccaactatgcgtgaggttctttggactcgatctggactccggtctattttctgcacccactgttccgttatccattaggaataatcactgggataactccccgtcgcctaacatgtacgggctgaataaagaagtggtccgtcagctctctcgcaggtacccacaactgcctcgggcagttgccactggaagagtctatgacatgaacactggtacactgcgcaattatgatccgcgcataaacctagtacctgtaaacagaagactgcctcatgctttagtcctccaccataatgaacacccacagagtgacttttcttcattcgtcagcaaattgaagggcagaactgtcctggtggtcggggaaaagttgtccgtcccaggcaaaatggttgactggttgtcagaccggcctgaggctaccttcagagctcggctggatttaggcatcccaggtgatgtgcccaaatatgacataatatttgttaatgtgaggaccccatataaataccatcactatcagcagtgtgaagaccatgccattaagcttagcatgttgaccaagaaagcttgtctgcatctgaatcccggcggaacctgtgtcagcataggttatggttacgctgacagggccagcgaaagcatcattggtgctatagcgcggcagttcaagttttcccgggtatgcaaaccgaaatcctcacttgaagagacggaagttctgtttgtattcattgggtacgatcgcaaggcccgtacgcacaatccttacaagctttcatcaaccttgaccaacatttatacaggttccagactccacgaagccggatgtgcaccctcatatcatgtggtgcgaggggatattgccacggccaccgaaggagtgattataaatgctgctaacagcaaaggacaacctggcggaggggtgtgcggagcgctgtataagaagttcccggaaagcttcgatttacagccgatcgaagtaggaaaagcgcgactggtcaaaggtgcagctaaacatatcattcatgccgtaggaccaaacttcaacaaagtttcggaggttgaaggtgacaaacagttggcagaggcttatgagtccatcgctaagattgtcaacgataacaattacaagtcagtagcgattccactgttgtccaccggcatcttttccgggaacaaagatcgactaacccaatcattgaaccatttgctgacagctttagacaccactgatgcagatgtagccatatactgcagggacaagaaatgggaaatgactctcaaggaagcagtggctaggagagaagcagtggaggagatatgcatatccgacgactcttcagtgacagaacctgatgcagagctggtgagggtgcatccgaagagttctttggctggaaggaagggctacagcacaagcgatggcaaaactttctcatatttggaagggaccaagtttcaccaggcggccaaggatatagcagaaattaatgccatgtggcccgttgcaacggaggccaatgagcaggtatgcatgtatatcctcggagaaagcatgagcagtattaggtcgaaatgccccgtcgaagagtcggaagcctcctcaccacctagcacgctgccttgcttgtgcatccatgccatgactccagaaagagtacagcgcctaaaagcctcacgtccagaacaaattactgtgtgctcatcctttccattgccgaagtatagaatcactggtgtgcagaagatccaatgctcccagcctatattgttctcaccgaaagtgcctgcgtatattcatccaaggaagtatctcgtggaaacaccaccggtagacgagactccggagccatcggcagagaaccaatccacagaggggacacctgaacaaccaccacttataaccgaggatgagaccaggactagaacgcctgagccgatcatcatcgaagaggaagaagaggatagcataagtttgctgtcagatggcccgacccaccaggtgctgcaagtcgaggcagacattcacgggccgccctctgtatctagctcatcctggtccattcctcatgcatccgactttgatgtggacagtttatccatacttgacaccctggagggagctagcgtgaccagcggggcaacgtcagccgagactaactcttacttcgcaaagagtatggagtttctggcgcgaccggtgcctgcgcctcgaacagtattcaggaaccctccacatcccgctccgcgcacaagaacaccgtcacttgcacccagcagggcctgctcgagaaccagcctagtttccaccccgccaggcgtgaatagggtgatcactagagaggagctcgaggcgcttaccccgtcacgcactcctagcaggtcggtctcgagaaccagcctggtctccaacccgccaggcgtaaatagggtgattacaagagaggagtttgaggcgttcgtagcacaacaacaatgacggtttgatgcgggtgcatacatcttttcctccgacaccggtcaagggcatttacaacaaaaatcagtaaggcaaacggtgctatccgaagtggtgttggagaggaccgaattggagatttcgtatgccccgcgcctcgaccaagaaaaagaagaattactacgcaagaaattacagttaaatcccacacctgctaacagaagcagataccagtccaggaaggtggagaacatgaaagccataacagctagacgtattctgcaaggcctagggcattatttgaaggcagaaggaaaagtggagtgctaccgaaccctgcatcctgttcctttgtattcatctagtgtgaaccgtgccttctcaagccccaaggtcgcagtggaagcctgtaacgccatgttgaaagagaactttccgactgtggcttcttactgtattattccagagtacgatgcctatttggacatggttgacggagcttcatgctgcttagacactgccagtttttgccctgcaaagctgcgcagctttccaaagaaacactcctatttggaacccacaatacgatcggcagtgccttcagcgatccagaacacgctccagaacgtcctggcagctgccacaaaaagaaattgcaatgtcacgcaaatgagagaattgcccgtattggattcggcggcctttaatgtggaatgcttcaagaaatatgcgtgtaataatgaatattgggaaacgtttaaagaaaaccccatcaggcttactgaagaaaacgtggtaaattacattaccaaattaaaaggaccaaaagctgctgctctttttgcgaagacacataatttgaatatgttgcaggacataccaatggacaggtttgtaatggacttaaagagagacgtgaaagtgactccaggaacaaaacatactgaagaacggcccaaggtacaggtgatccaggctgccgatccgctagcaacagcgtatctgtgcggaatccaccgagagctggttaggagattaaatgcggtcctgcttccgaacattcatacactgtttgatatgtcggctgaagactttgacgctattatagccgagcacttccagcctggggattgtgttctggaaactgacatcgcgtcgtttgataaaagtgaggacgacgccatggctctgaccgcgttaatgattctggaagacttaggtgtggacgcagagctgttgacgctgattgaggcggctttcggcgaaatttcatcaatacatttgcccactaaaactaaatttaaattcggagccatgatgaaatctggaatgttcctcacactgtttgtgaacacagtcattaacattgtaatcgcaagcagagtgttgagagaacggctaaccggatcaccatgtgcagcattcattggagatgacaatatcgtgaaaggagtcaaatcggacaaattaatggcagacaggtgcgccacctggttgaatatggaagtcaagattatagatgctgtggtgggcgagaaagcgccctatttctgtggagggtttattttgtgtgactccgtgaccggcacagcgtgccgtgtggcagaccccctaaaaaggctgtttaagcttggcaaacctctggcagcagacgatgaacatgatgatgacaggagaagggcattgcatgaagagtcaacacgctggaaccgagtgggtattctttcagagctgtgcaaggcagtagaatcaaggtatgaaaccgtaggaacttccatcatagttatggccatgactactctagctagcagtgttaaatcattcagctacctgagaggggcccctataactctctacggctaacctgaatggactacgacatcgatggcgcgccaccatggtgagcaagggcgaggagctgttcaccggggtggtgcccatcctggtcgagctggacggcgacgtaaacggccacaagttcagcgtgtccggcgagggcgagggcgatgccacctacggcaagctgaccctgaagttcatctgcaccaccggcaagctgcccgtgccctggcccaccctcgtgaccaccctgacctacggcgtgcagtgcttcagccgctaccccgaccacatgaagcagcacgacttcttcaagtccgccatgcccgaaggctacgtccaggagcgcaccatcttcttcaaggacgacggcaactacaagacccgcgccgaggtgaagttcgagggcgacaccctggtgaaccgcatcgagctgaagggcatcgacttcaaggaggacggcaacatcctggggcacaagctggagtacaactacaacagccacaacgtctatatcatggccgacaagcagaagaacggcatcaaggtgaacttcaagatccgccacaacatcgaggacggcagcgtgcagctcgccgaccactaccagcagaacacccccatcggcgacggccccgtgctgctgcccgacaaccactacctgagcacccagtccgccctgagcaaagaccccaacgagaagcgcgatcacatggtcctgctggagttcgtgaccgccgccgggatcactctcggcatggacgagctgtacaaggctagcatcgagggccggggcggctggggcaaagagacagccgccgccaagttcgagcggcagcacatggacagctgataattaattaagtaaccgatacagcagcaattggcaagctgcttacatagaactcgcggcgattggcatgccgctttaaaatttttattttattttttcttttcttttccgaatcggattttgtttttaatatttcaaaaaaaaaaaaaaaaaaaaaaaaaaaaaaaaaaaaaaaaaaaaaaaaaaggaagagcgcggccgcatccggcgttcagcctgtgccacagccgacaggatggtgaccaccatttgccccatatcaccgtcggtactgatcccgtcgtcaataaaccgaaccgctacaccctgagcatcaaactcttttatcagttggatcatgtcggcggtgtcgcggccaagacggtcgagcttcttcaccagaatgacatcaccttcctccaccttcatcctcagcaaatccagcccttcccgatctgttgaactgccggatgccttgtcggtaaagatgcggttagcttttacccctgcatctttgagcgctgaggtctgcctcgtgaagaaggtgttgctgactcataccaggcctgaatcgccccatcatccagccagaaagtgagggagccacggttgatgagagctttgttgtaggtggaccagttggtgattttgaacttttgctttgccacggaacggtctgcgttgtcgggaagatgcgtgatctgatccttcaactcagcaaaagttcgatttattcaacaaagccgccgtcccgtcaagtcagcgtaatgctctgccagtgttacaaccaattaaccaattctgattagaaaaactcatcgagcatcaaatgaaactgcaatttattcatatcaggattatcaataccatatttttgaaaaagccgtttctgtaatgaaggagaaaactcaccgaggcagttccataggatggcaagatcctggtatcggtctgcgattccgactcgtccaacatcaatacaacctattaatttcccctcgtcaaaaataaggttatcaagtgagaaatcaccatgagtgacgactgaatccggtgagaatggcaaaagcttatgcatttctttccagacttgttcaacaggccagccattacgctcgtcatcaaaatcactcgcatcaaccaaaccgttattcattcgtgattgcgcctgagcgagacgaaatacgcgatcgctgttaaaaggacaattacaaacaggaatcgaatgcaaccggcgcaggaacactgccagcgcatcaacaatattttcacctgaatcaggatattcttctaatacctggaatgctgttttcccggggatcgcagtggtgagtaaccatgcatcatcaggagtacggataaaatgcttgatggtcggaagaggcataaattccgtcagccagtttagtctgaccatctcatctgtaacatcattggcaacgctacctttgccatgtttcagaaacaactctggcgcatcgggcttcccatacaatcgatagattgtcgcacctgattgcccgacattatcgcgagcccatttatacccatataaatcagcatccatgttggaatttaatcgcggcctcgagcaagacgtttcccgttgaatatggctcataacaccccttgtattactgtttatgtaagcagacagttttattgttcatgatgatatatttttatcttgtgcaatgtaacatcagagattttgagacacaacgtggctttgttgaataaatcgaacttttgctgagttgaaggatcagatcacgcatcttcccgacaacgcagaccgttccgtggcaaagcaaaagttcaaaatcaccaactggtccacctacaacaaagctctcatcaaccgtggctccctcactttctggctggatgatggggcgattcaggcctggtatgagtcagcaacaccttcttcacgaggcagacctcagcgctagcggagtgtatactggcttactatgttggcactgatgagggtgtcagtgaagtgcttcatgtggcaggagaaaaaaggctgcaccggtgcgtcagcagaatatgtgatacaggatatattccgcttcctcgctcactgactcgctacgctcggtcgttcgactgcggcgagcggaaatggcttacgaacggggcggagatttcctggaagatgccaggaagatacttaacagggaagtgagagggccgcggcaaagccgtttttccataggctccgcccccctgacaagcatcacgaaatctgacgctcaaatcagtggtggcgaaacccgacaggactataaagataccaggcgtttccccctggcggctccctcgtgcgctctcctgttcctgcctttcggtttaccggtgtcattccgctgttatggccgcgtttgtctcattccacgcctgacactcagttccgggtaggcagttcgctccaagctggactgtatgcacgaaccccccgttcagtccgaccgctgcgccttatccggtaactatcgtcttgagtccaacccggaaagacatgcaaaagcaccactggcagcagccactggtaattgatttagaggagttagtcttgaagtcatgcgccggttaaggctaaactgaaaggacaagttttggtgactgcgctcctccaagccagttacctcggttcaaagagttggtagctcagagaaccttcgaaaaaccgccctgcaaggcggttttttcgttttcagagcaagagattacgcgcagaccaaaacgatctcaagaagatcatcttattaaggggtctgacgctcagtggaacgaaaactcacgttaagggattttggtcatgagattatcaaaaaggatcttcacctagatccttttaaattaaaaatgaagttttaaatcaatctaaagtatatatgagtaaacttggtctgacagttaccaatgcttaatcagtgaggcacctatctcagcgatctgtctatttcgttcatccatagttgcctgactccccgtcgtgtagataactacgatacgggagggcttaccatctggccccagtgctgcaatgataccgcgagacccacgctcaccggctccagatttatcagcaataaaccagccagccggaagggccgagcgcagaagtggtcctgcaactttatccgcctccatccagtctattaattgttgccgggaagctagagtaagtagttcgccagttaatagtttgcgcaacgttgttgccattgctgcaggcatcgtggtgtcacgctcgtcgtttggtatggcttcattcagctccggttcccaacgatcaaggcgagttacatgatcccccatgttgtgcaaaaaagcggttagctccttcggtcctccgatcgttgtcagaagtaagttggccgcagtgttatcactcatggttatggcagcactgcataattctcttactgtcatgccatccgtaagatgcttttctgtgactggtgagtactcaaccaagtcattctgagaatagtgtatgcggcgaccgagttgctcttgcccggcgtcaacacgggataataccgcgccacatagcagaactttaaaagtgctcatcattggaaaacgttcttcggggcgaaaactctcaaggatcttaccgctgttgagatccagttcgatgtaacccactcgtgcacccaactgatcttcagcatcttttactttcaccagcgtttctgggtgagcaaaaacaggaaggcaaaatgccgcaaaaaagggaataagggcgacacggaaatgttgaatactcatactcttcctttttcaatattattgaagcatttatcagggttattgtctcatgagcggatacatatttgaatgtatttagaaaaataaacaaataggggttccgcgcacatttccccgaaaagtgccacctgacgtctaagaaaccattattatcatgacattaacctataaaaataggcgtatcacgaggccctttcgtcttcaagaatttctagaggatccctaatacgactcactatag

SEQ ID NO: 2 - DNA, 4003 bp, synthetic construct
  source 1..4003: mol_type = other DNA
ttaattaagtaaccgatacagcagcaattggcaagctgcttacatagaactcgcggcgattggcatgccgctttaaaatttttattttattttttcttttcttttccgaatcggattttgtttttaatatttcaaaaaaaaaaaaaaaaaaaaaaaaaaaaaaaaaaaaaaaaaaaaaaaaaaggaagagcgcggccgcatccggcgttcagcctgtgccacagccgacaggatggtgaccaccatttgccccatatcaccgtcggtactgatcccgtcgtcaataaaccgaaccgctacaccctgagcatcaaactcttttatcagttggatcatgtcggcggtgtcgcggccaagacggtcgagcttcttcaccagaatgacatcaccttcctccaccttcatcctcagcaaatccagcccttcccgatctgttgaactgccggatgccttgtcggtaaagatgcggttagcttttacccctgcatctttgagcgctgaggtctgcctcgtgaagaaggtgttgctgactcataccaggcctgaatcgccccatcatccagccagaaagtgagggagccacggttgatgagagctttgttgtaggtggaccagttggtgattttgaacttttgctttgccacggaacggtctgcgttgtcgggaagatgcgtgatctgatccttcaactcagcaaaagttcgatttattcaacaaagccgccgtcccgtcaagtcagcgtaatgctctgccagtgttacaaccaattaaccaattctgattagaaaaactcatcgagcatcaaatgaaactgcaatttattcatatcaggattatcaataccatatttttgaaaaagccgtttctgtaatgaaggagaaaactcaccgaggcagttccataggatggcaagatcctggtatcggtctgcgattccgactcgtccaacatcaatacaacctattaatttcccctcgtcaaaaataaggttatcaagtgagaaatcaccatgagtgacgactgaatccggtgagaatggcaaaagcttatgcatttctttccagacttgttcaacaggccagccattacgctcgtcatcaaaatcactcgcatcaaccaaaccgttattcattcgtgattgcgcctgagcgagacgaaatacgcgatcgctgttaaaaggacaattacaaacaggaatcgaatgcaaccggcgcaggaacactgccagcgcatcaacaatattttcacctgaatcaggatattcttctaatacctggaatgctgttttcccggggatcgcagtggtgagtaaccatgcatcatcaggagtacggataaaatgcttgatggtcggaagaggcataaattccgtcagccagtttagtctgaccatctcatctgtaacatcattggcaacgctacctttgccatgtttcagaaacaactctggcgcatcgggcttcccatacaatcgatagattgtcgcacctgattgcccgacattatcgcgagcccatttatacccatataaatcagcatccatgttggaatttaatcgcggcctcgagcaagacgtttcccgttgaatatggctcataacaccccttgtattactgtttatgtaagcagacagttttattgttcatgatgatatatttttatcttgtgcaatgtaacatcagagattttgagacacaacgtggctttgttgaataaatcgaacttttgctgagttgaaggatcagatcacgcatcttcccgacaacgcagaccgttccgtggcaaagcaaaagttcaaaatcaccaactggtccacctacaacaaagctctcatcaaccgtggctccctcactttctggctggatgatggggcgattcaggcctggtatgagtcagcaacaccttcttcacgaggcagacctcagcgctagcggagtgtatactggcttactatgttggcactgatgagggtgtcagtgaagtgcttcatgtggcaggagaaaaaaggctgcaccggtgcgtcagcagaatatgtgatacaggatatattccgcttcctcgctcactgactcgctacgctcggtcgttcgactgcggcgagcggaaatggcttacgaacggggcggagatttcctggaagatgccaggaagatacttaacagggaagtgagagggccgcggcaaagccgtttttccataggctccgcccccctgacaagcatcacgaaatctgacgctcaaatcagtggtggcgaaacccgacaggactataaagataccaggcgtttccccctggcggctccctcgtgcgctctcctgttcctgcctttcggtttaccggtgtcattccgctgttatggccgcgtttgtctcattccacgcctgacactcagttccgggtaggcagttcgctccaagctggactgtatgcacgaaccccccgttcagtccgaccgctgcgccttatccggtaactatcgtcttgagtccaacccggaaagacatgcaaaagcaccactggcagcagccactggtaattgatttagaggagttagtcttgaagtcatgcgccggttaaggctaaactgaaaggacaagttttggtgactgcgctcctccaagccagttacctcggttcaaagagttggtagctcagagaaccttcgaaaaaccgccctgcaaggcggttttttcgttttcagagcaagagattacgcgcagaccaaaacgatctcaagaagatcatcttattaaggggtctgacgctcagtggaacgaaaactcacgttaagggattttggtcatgagattatcaaaaaggatcttcacctagatccttttaaattaaaaatgaagttttaaatcaatctaaagtatatatgagtaaacttggtctgacagttaccaatgcttaatcagtgaggcacctatctcagcgatctgtctatttcgttcatccatagttgcctgactccccgtcgtgtagataactacgatacgggagggcttaccatctggccccagtgctgcaatgataccgcgagacccacgctcaccggctccagatttatcagcaataaaccagccagccggaagggccgagcgcagaagtggtcctgcaactttatccgcctccatccagtctattaattgttgccgggaagctagagtaagtagttcgccagttaatagtttgcgcaacgttgttgccattgctgcaggcatcgtggtgtcacgctcgtcgtttggtatggcttcattcagctccggttcccaacgatcaaggcgagttacatgatcccccatgttgtgcaaaaaagcggttagctccttcggtcctccgatcgttgtcagaagtaagttggccgcagtgttatcactcatggttatggcagcactgcataattctcttactgtcatgccatccgtaagatgcttttctgtgactggtgagtactcaaccaagtcattctgagaatagtgtatgcggcgaccgagttgctcttgcccggcgtcaacacgggataataccgcgccacatagcagaactttaaaagtgctcatcattggaaaacgttcttcggggcgaaaactctcaaggatcttaccgctgttgagatccagttcgatgtaacccactcgtgcacccaactgatcttcagcatcttttactttcaccagcgtttctgggtgagcaaaaacaggaaggcaaaatgccgcaaaaaagggaataagggcgacacggaaatgttgaatactcatactcttcctttttcaatattattgaagcatttatcagggttattgtctcatgagcggatacatatttgaatgtatttagaaaaataaacaaataggggttccgcgcacatttccccgaaaagtgccacctgacgtctaagaaaccattattatcatgacattaacctataaaaataggcgtatcacgaggccctttcgtcttcaagaatttctagaggatccctaatacgactcactatag

SEQ ID NO: 3 - DNA, 7560 bp, synthetic construct
  source 1..7560: mol_type = other DNA
atgggcggcgcatgagagaagcccagaccaattacctacccaaaatggagaaagttcacgttgacatcgaggaagacagcccattcctcagagctttgcagcggagcttcccgcagtttgaggtagaagccaagcaggtcactgataatgaccatgctaatgccagagcgttttcgcatctggcttcaaaactgatcgaaacggaggtggacccatccgacacgatccttgacattggaagtgcgcccgcccgcagaatgtattctaagcacaagtatcattgtatctgtccgatgagatgtgcggaagatccggacagattgtataagtatgcaactaagctgaagaaaaactgtaaggaaataactgataaggaattggacaagaaaatgaaggagctcgccgccgtcatgagcgaccctgacctggaaactgagactatgtgcctccacgacgacgagtcgtgtcgctacgaagggcaagtcgctgtttaccaggatgtatacgcggttgacggaccgacaagtctctatcaccaagccaataagggagttagagtcgcctactggataggctttgacaccaccccttttatgtttaagaacttggctggagcatatccatcatactctaccaactgggccgacgaaaccgtgttaacggctcgtaacataggcctatgcagctctgacgttatggagcggtcacgtagagggatgtccattcttagaaagaagtatttgaaaccatccaacaatgttctattctctgttggctcgaccatctaccacgagaagagggacttactgaggagctggcacctgccgtctgtatttcacttacgtggcaagcaaaattacacatgtcggtgtgagactatagttagttgcgacgggtacgtcgttaaaagaatagctatcagtccaggcctgtatgggaagccttcaggctatgctgctacgatgcaccgcgagggattcttgtgctgcaaagtgacagacacattgaacggggagagggtctcttttcccgtgtgcacgtatgtgccagctacattgtgtgaccaaatgactggcatactggcaacagatgtcagtgcggacgacgcgcaaaaactgctggttgggctcaaccagcgtatagtcgtcaacggtcgcacccagagaaacaccaataccatgaaaaattaccttttgcccgtagtggcccaggcatttgctaggtgggcaaaggaatataaggaagatcaagaagatgaaaggccactaggactacgagatagacagttagtcatggggtgttgttgggcttttagaaggcacaagataacatctatttataagcgcccggatacccaaaccatcatcaaagtgaacagcgatttccactcattcgtgctgcccaggataggcagtaacacattggagatcgggctgagaacaagaatcaggaaaatgttagaggagcacaaggagccgtcacctctcattaccgccgaggacgtacaagaagctaagtgcgcagccgatgaggctaaggaggtgcgtgaagccgaggagttgcgcgcagctctaccacctttggcagctgatgttgaggagcccactctggaagccgatgtcgacttgatgttacaagaggctggggccggctcagtggagacacctcgtggcttgataaaggttaccagctacgctggcgaggacaagatcggctcttacgctgtgctttctccgcaggctgtactcaagagtgaaaaattatcttgcatccaccctctcgctgaacaagtcatagtgataacacactctggccgaaaagggcgttatgccgtggaaccataccatggtaaagtagtggtgccagagggacatgcaatacccgtccaggactttcaagctctgagtgaaagtgccaccattgtgtacaacgaacgtgagttcgtaaacaggtacctgcaccatattgccacacatggaggagcgctgaacactgatgaagaatattacaaaactgtcaagcccagcgagcacgacggcgaatacctgtacgacatcgacaggaaacagtgcgtcaagaaagaactagtcactgggctagggctcacaggcgagctggtggatcctcccttccatgaattcgcctacgagagtctgagaacacgaccagccgctccttaccaagtaccaaccataggggtgtatggcgtgccaggatcaggcaagtctggcatcattaaaagcgcagtcaccaaaaaagatctagtggtgagcgccaagaaagaaaactgtgcagaaattataagggacgtcaagaaaatgaaagggctggacgtcaatgccagaactgtggactcagtgctcttgaatggatgcaaacaccccgtagagaccctgtatattgacgaagcttttgcttgtcatgcaggtactctcagagcgctcatagccattataagacctaaaaaggcagtgctctgcggggatcccaaacagtgcggtttttttaacatgatgtgcctgaaagtgcattttaaccacgagatttgcacacaagtcttccacaaaagcatctctcgccgttgcactaaatctgtgacttcggtcgtctcaaccttgttttacgacaaaaaaatgagaacgacgaatccgaaagagactaagattgtgattgacactaccggcagtaccaaacctaagcaggacgatctcattctcacttgtttcagagggtgggtgaagcagttgcaaatagattacaaaggcaacgaaataatgacggcagctgcctctcaagggctgacccgtaaaggtgtgtatgccgttcggtacaaggtgaatgaaaatcctctgtacgcacccacctcagaacatgtgaacgtcctactgacccgcacggaggaccgcatcgtgtggaaaacactagccggcgacccatggataaaaacactgactgccaagtaccctgggaatttcactgccacgatagaggagtggcaagcagagcatgatgccatcatgaggcacatcttggagagaccggaccctaccgacgtcttccagaataaggcaaacgtgtgttgggccaaggctttagtgccggtgctgaagaccgctggcatagacatgaccactgaacaatggaacactgtggattattttgaaacggacaaagctcactcagcagagatagtattgaaccaactatgcgtgaggttctttggactcgatctggactccggtctattttctgcacccactgttccgttatccattaggaataatcactgggataactccccgtcgcctaacatgtacgggctgaataaagaagtggtccgtcagctctctcgcaggtacccacaactgcctcgggcagttgccactggaagagtctatgacatgaacactggtacactgcgcaattatgatccgcgcataaacctagtacctgtaaacagaagactgcctcatgctttagtcctccaccataatgaacacccacagagtgacttttcttcattcgtcagcaaattgaagggcagaactgtcctggtggtcggggaaaagttgtccgtcccaggcaaaatggttgactggttgtcagaccggcctgaggctaccttcagagctcggctggatttaggcatcccaggtgatgtgcccaaatatgacataatatttgttaatgtgaggaccccatataaataccatcactatcagcagtgtgaagaccatgccattaagcttagcatgttgaccaagaaagcttgtctgcatctgaatcccggcggaacctgtgtcagcataggttatggttacgctgacagggccagcgaaagcatcattggtgctatagcgcggcagttcaagttttcccgggtatgcaaaccgaaatcctcacttgaagagacggaagttctgtttgtattcattgggtacgatcgcaaggcccgtacgcacaatccttacaagctttcatcaaccttgaccaacatttatacaggttccagactccacgaagccggatgtgcaccctcatatcatgtggtgcgaggggatattgccacggccaccgaaggagtgattataaatgctgctaacagcaaaggacaacctggcggaggggtgtgcggagcgctgtataagaagttcccggaaagcttcgatttacagccgatcgaagtaggaaaagcgcgactggtcaaaggtgcagctaaacatatcattcatgccgtaggaccaaacttcaacaaagtttcggaggttgaaggtgacaaacagttggcagaggcttatgagtccatcgctaagattgtcaacgataacaattacaagtcagtagcgattccactgttgtccaccggcatcttttccgggaacaaagatcgactaacccaatcattgaaccatttgctgacagctttagacaccactgatgcagatgtagccatatactgcagggacaagaaatgggaaatgactctcaaggaagcagtggctaggagagaagcagtggaggagatatgcatatccgacgactcttcagtgacagaacctgatgcagagctggtgagggtgcatccgaagagttctttggctggaaggaagggctacagcacaagcgatggcaaaactttctcatatttggaagggaccaagtttcaccaggcggccaaggatatagcagaaattaatgccatgtggcccgttgcaacggaggccaatgagcaggtatgcatgtatatcctcggagaaagcatgagcagtattaggtcgaaatgccccgtcgaagagtcggaagcctcctcaccacctagcacgctgccttgcttgtgcatccatgccatgactccagaaagagtacagcgcctaaaagcctcacgtccagaacaaattactgtgtgctcatcctttccattgccgaagtatagaatcactggtgtgcagaagatccaatgctcccagcctatattgttctcaccgaaagtgcctgcgtatattcatccaaggaagtatctcgtggaaacaccaccggtagacgagactccggagccatcggcagagaaccaatccacagaggggacacctgaacaaccaccacttataaccgaggatgagaccaggactagaacgcctgagccgatcatcatcgaagaggaagaagaggatagcataagtttgctgtcagatggcccgacccaccaggtgctgcaagtcgaggcagacattcacgggccgccctctgtatctagctcatcctggtccattcctcatgcatccgactttgatgtggacagtttatccatacttgacaccctggagggagctagcgtgaccagcggggcaacgtcagccgagactaactcttacttcgcaaagagtatggagtttctggcgcgaccggtgcctgcgcctcgaacagtattcaggaaccctccacatcccgctccgcgcacaagaacaccgtcacttgcacccagcagggcctgctcgagaaccagcctagtttccaccccgccaggcgtgaatagggtgatcactagagaggagctcgaggcgcttaccccgtcacgcactcctagcaggtcggtctcgagaaccagcctggtctccaacccgccaggcgtaaatagggtgattacaagagaggagtttgaggcgttcgtagcacaacaacaatgacggtttgatgcgggtgcatacatcttttcctccgacaccggtcaagggcatttacaacaaaaatcagtaaggcaaacggtgctatccgaagtggtgttggagaggaccgaattggagatttcgtatgccccgcgcctcgaccaagaaaaagaagaattactacgcaagaaattacagttaaatcccacacctgctaacagaagcagataccagtccaggaaggtggagaacatgaaagccataacagctagacgtattctgcaaggcctagggcattatttgaaggcagaaggaaaagtggagtgctaccgaaccctgcatcctgttcctttgtattcatctagtgtgaaccgtgccttctcaagccccaaggtcgcagtggaagcctgtaacgccatgttgaaagagaactttccgactgtggcttcttactgtattattccagagtacgatgcctatttggacatggttgacggagcttcatgctgcttagacactgccagtttttgccctgcaaagctgcgcagctttccaaagaaacactcctatttggaacccacaatacgatcggcagtgccttcagcgatccagaacacgctccagaacgtcctggcagctgccacaaaaagaaattgcaatgtcacgcaaatgagagaattgcccgtattggattcggcggcctttaatgtggaatgcttcaagaaatatgcgtgtaataatgaatattgggaaacgtttaaagaaaaccccatcaggcttactgaagaaaacgtggtaaattacattaccaaattaaaaggaccaaaagctgctgctctttttgcgaagacacataatttgaatatgttgcaggacataccaatggacaggtttgtaatggacttaaagagagacgtgaaagtgactccaggaacaaaacatactgaagaacggcccaaggtacaggtgatccaggctgccgatccgctagcaacagcgtatctgtgcggaatccaccgagagctggttaggagattaaatgcggtcctgcttccgaacattcatacactgtttgatatgtcggctgaagactttgacgctattatagccgagcacttccagcctggggattgtgttctggaaactgacatcgcgtcgtttgataaaagtgaggacgacgccatggctctgaccgcgttaatgattctggaagacttaggtgtggacgcagagctgttgacgctgattgaggcggctttcggcgaaatttcatcaatacatttgcccactaaaactaaatttaaattcggagccatgatgaaatctggaatgttcctcacactgtttgtgaacacagtcattaacattgtaatcgcaagcagagtgttgagagaacggctaaccggatcaccatgtgcagcattcattggagatgacaatatcgtgaaaggagtcaaatcggacaaattaatggcagacaggtgcgccacctggttgaatatggaagtcaagattatagatgctgtggtgggcgagaaagcgccctatttctgtggagggtttattttgtgtgactccgtgaccggcacagcgtgccgtgtggcagaccccctaaaaaggctgtttaagcttggcaaacctctggcagcagacgatgaacatgatgatgacaggagaagggcattgcatgaagagtcaacacgctggaaccgagtgggtattctttcagagctgtgcaaggcagtagaatcaaggtatgaaaccgtaggaacttccatcatagttatggccatgactactctagctagcagtgttaaatcattcagctacctgagaggggcccctataactctctacggctaacctgaatggactacgacatcgatggcgcgccacc

SEQ ID NO: 4 - DNA, 717 bp, synthetic construct
  source 1..717: mol_type = other DNA
atggtgagcaagggcgaggagctgttcaccggggtggtgcccatcctggtcgagctggacggcgacgtaaacggccacaagttcagcgtgtccggcgagggcgagggcgatgccacctacggcaagctgaccctgaagttcatctgcaccaccggcaagctgcccgtgccctggcccaccctcgtgaccaccctgacctacggcgtgcagtgcttcagccgctaccccgaccacatgaagcagcacgacttcttcaagtccgccatgcccgaaggctacgtccaggagcgcaccatcttcttcaaggacgacggcaactacaagacccgcgccgaggtgaagttcgagggcgacaccctggtgaaccgcatcgagctgaagggcatcgacttcaaggaggacggcaacatcctggggcacaagctggagtacaactacaacagccacaacgtctatatcatggccgacaagcagaagaacggcatcaaggtgaacttcaagatccgccacaacatcgaggacggcagcgtgcagctcgccgaccactaccagcagaacacccccatcggcgacggccccgtgctgctgcccgacaaccactacctgagcacccagtccgccctgagcaaagaccccaacgagaagcgcgatcacatggtcctgctggagttcgtgaccgccgccgggatcactctcggcatggacgagctgtacaag

SEQ ID NO: 5 - DNA, 7691 bp, synthetic construct
  source 1..7691: mol_type = other DNA
gtcgacattgattattgactagttattaatagtaatcaattacggggtcattagttcatagcccatatatggagttccgcgttacataacttacggtaaatggcccgcctggctgaccgcccaacgacccccgcccattgacgtcaataatgacgtatgttcccatagtaacgccaatagggactttccattgacgtcaatgggtggactatttacggtaaactgcccacttggcagtacatcaagtgtatcatatgccaagtacgccccctattgacgtcaatgacggtaaatggcccgcctggcattatgcccagtacatgaccttatgggactttcctacttggcagtacatctacgtattagtcatcgctattaccatgggtcgaggtgagccccacgttctgcttcactctccccatctcccccccctccccacccccaattttgtatttatttattttttaattattttgtgcagcgatgggggcggggggggggggggcgcgcgccaggcggggcggggcggggcgaggggcggggcggggcgaggcggagaggtgcggcggcagccaatcagagcggcgcgctccgaaagtttccttttatggcgaggcggcggcggcggcggccctataaaaagcgaagcgcgcggcgggcgggagtcgctgcgttgccttcgccccgtgccccgctccgcgccgcctcgcgccgcccgccccggctctgactgaccgcgttactcccacaggtgagcgggcgggacggcccttctcctccgggctgtaattagcgcttggtttaatgacggctcgtttcttttctgtggctgcgtgaaagccttaaagggctccgggagggccctttgtgcgggggggagcggctcggggggtgcgtgcgtgtgtgtgtgcgtggggagcgccgcgtgcggcccgcgctgcccggcggctgtgagcgctgcgggcgcggcgcggggctttgtgcgctccgcgtgtgcgcgaggggagcgcggccgggggcggtgccccgcggtgcgggggggctgcgaggggaacaaaggctgcgtgcggggtgtgtgcgtgggggggtgagcagggggtgtgggcgcggcggtcgggctgtaacccccccctgcacccccctccccgagttgctgagcacggcccggcttcgggtgcggggctccgtgcggggcgtggcgcggggctcgccgtgccgggcggggggtggcggcaggtgggggtgccgggcggggcggggccgcctcgggccggggagggctcgggggaggggcgcggcggccccggagcgccggcggctgtcgaggcgcggcgagccgcagccattgccttttatggtaatcgtgcgagagggcgcagggacttcctttgtcccaaatctgtgcggagccgaaatctgggaggcgccgccgcaccccctctagcgggcgcggggcgaagcggtgcggcgccggcaggaaggaaatgggcggggagggccttcgtgcgtcgccgcgccgccgtccccttctccctctccagcctcggggctgtccgcggggggacggctgccttcgggggggacggggcagggcggggttcggcttctggcgtgtgaccggcggctctagagcctctgctaaccatgttcatgccttcttctttttcctacagctcctgggcaacgtgctggttattgtgctgtctcatcattttggcaaagaattcggcggccgcatgagtctggccattccagttatgtgcctgctggcaaataccacgttcccctgctcccagcccccttgcacaccctgctgctacgaaaaagagccggagaaaaccttgcgcatgcttgaagacaatgtcatgagccccgggtactatcagctgctacaagcatccttaacatgttctccccgacgccagcggcgcagtattaaggaccacttcaatgtctataaagccacaagaccgtacctagctcactgtcccgactgtggagaagggcactcgtgccatagtcccgtagcgctagaacgcatcagaaacgaagcgacagacgggacgttgaaaatccaggtttccttgcaaatcggaataaagacggatgatagccatgattggaccaagctgcgttatatggacaatcacatgccagcagacgcagagcgggccgggctatttgtaagaacgtcagcaccgtgcacgattactggaacaatgggacacttcattctggcccgatgtccgaaaggagaaactctgacggtagggttcactgacggtaggaagatcagtcactcatgtacgcacccatttcaccatgaccctcctgtgataggccgggaaaaattccattcccgaccgcagcacggtagggaactaccttgcagcacgtacgcgcagagcaccgctgcaactgccgaggagatagaggtacatatgcccccagacaccccagatcgcacattaatgtcacaacagtccggcaatgtaaagatcacagtcaatagtcagacggtgcggtacaagtgcaattgtggtgactcaagtgaaggattaaccactacagataaagtgattaataactgcaaggttgatcaatgccatgccgcggtcaccaatcacaaaaaatggcagtataattcccctctggtcccgcgtaatgctgaattcggggaccggaaaggaaaagttcacattccatttcctctggcaaatgtgacatgcagggtgcctaaagcaagaaaccccaccgtgacgtacggaaaaaaccaagtcatcatgttgctgtatcctgaccacccaacgctcctgtcctacaggaatatgggagaagaaccaaactatcaagaagagtgggtgacgcataagaaggagatcaggttaaccgtgccgactgaagggctcgaggtcacgtggggtaacaatgagccgtacaagtattggccgcagttatccacaaacggtacagcccacggccacccgcatgagataattctgtattattatgagctgtacccaactatgactgtggtagttttgtcagtggcctcgttcatactcctgtcgatggtgggtgtggcagtggggatgtgcatgtgtgcacgacgcagatgcattacaccgtacgaactgacaccaggagctaccgtccctttcctgcttagcctaatatgctgcattagaacagctaaagcggccacataccaggaggccgcggtatacctgtggaacgagcagcagcctttattttggctgcaagcccttattccgctggcagccctgattgtcctatgtaactgtctgagactcttaccatgctgttgtaaaatgttgacttttttagccgtactgagcgtcggtgcccacactgtgagtgcgtacgaacacgtaacagtgatcccgaacacggtgggagtaccgtataagactctagtcaacagaccgggctacagccccatggtattggagatggagcttctgtctgtcaccttggaaccaacgctatcgcttgattacatcacgtgcgagtataaaaccgttatcccgtctccgtacgtgaaatgctgcggtacagcagagtgtaaggacaagagcctacctgattacagctgtaaggtcttcaccggcgtctacccattcatgtggggcggcgcctactgcttctgcgacaccgaaaatacgcaattgagcgaagcacatgtggagaagtccgaatcatgcaaaacagaatttgcatcagcatacagggctcataccgcatccgcgtcagctaagctccgcgtcctttaccaaggaaataatatcactgtagctgcttatgcaaacggcgaccatgccgtcacagttaaggacgctaaattcatagtggggccaatgtcttcagcctggacacctttcgacaataaaatcgtggtgtacaaaggcgacgtctacaacatggactacccgcccttcggcgcaggaagaccaggacaatttggcgacatccaaagtcgcacgcctgagagcgaagacgtctatgctaatacacaactggtactgcagagaccgtccgcgggtacggtgcacgtgccgtactctcaggcaccatctggcttcaagtattggctaaaagaacgaggggcgtcgctgcagcacacagcaccatttggctgtcaaatagcaacaaacccggtaagagcgatgaactgcgccgtagggaacatgcctatctccatcgacataccggacgcggcctttaccagggtcgtcgacgcgccatctttaacggacatgtcgtgtgaggtatcagcctgcacccattcctcagactttgggggcgtagccatcattaaatatgcagccagtaagaaaggcaagtgtgcagtgcactcgatgactaacgccgtcactattcgggaagctgaaatagaagtagaagggaactctcagttgcaaatctctttttcgacggccctagccagcgccgaatttcgcgtacaagtctgttctacacaagtacactgtgcagccgagtgccatccaccgaaagaccatatagtcaattacccggcgtcacacaccaccctcggggtccaagacatttccgctacggcgatgtcatgggtgcagaagatcacgggaggtgtgggactggttgtcgctgttgcagcactgatcctaatcgtggtgctatgcgtgtcgtttagcaggcactaagctagcagatctttttccctctgccaaaaattatggggacatcatgaagccccttgagcatctgacttctggctaataaaggaaatttattttcattgcaatagtgtgttggaattttttgtgtctctcactcggaaggacatatgggagggcaaatcatttaaaacatcagaatgagtatttggtttagagtttggcaacatatgcccatatgctggctgccatgaacaaaggttggctataaagaggtcatcagtatatgaaacagccccctgctgtccattccttattccatagaaaagccttgacttgaggttagattttttttatattttgttttgtgttatttttttctttaacatccctaaaattttccttacatgttttactagccagatttttcctcctctcctgactactcccagtcatagctgtccctcttctcttatggagatccctcgacctgcagcccaagcttggcgtaatcatggtcatagctgtttcctgtgtgaaattgttatccgctcacaattccacacaacatacgagccggaagcataaagtgtaaagcctggggtgcctaatgagtgagctaactcacattaattgcgttgcgctcactgcccgctttccagtcgggaaacctgtcgtgccagcggatccgcatctcaattagtcagcaaccatagtcccgcccctaactccgcccatcccgcccctaactccgcccagttccgcccattctccgccccatggctgactaattttttttatttatgcagaggccgaggccgcctcggcctctgagctattccagaagtagtgaggaggcttttttggaggcctaggcttttgcaaaaagctaacttgtttattgcagcttataatggttacaaataaagcaatagcatcacaaatttcacaaataaagcatttttttcactgcattctagttgtggtttgtccaaactcatcaatgtatcttatcatgtctggatccgctgcattaatgaatcggccaacgcgcggggagaggcggtttgcgtattgggcgctcttccgcttcctcgctcactgactcgctgcgctcggtcgttcggctgcggcgagcggtatcagctcactcaaaggcggtaatacggttatccacagaatcaggggataacgcaggaaagaacatgtgagcaaaaggccagcaaaaggccaggaaccgtaaaaaggccgcgttgctggcgtttttccataggctccgcccccctgacgagcatcacaaaaatcgacgctcaagtcagaggtggcgaaacccgacaggactataaagataccaggcgtttccccctggaagctccctcgtgcgctctcctgttccgaccctgccgcttaccggatacctgtccgcctttctcccttcgggaagcgtggcgctttctcaatgctcacgctgtaggtatctcagttcggtgtaggtcgttcgctccaagctgggctgtgtgcacgaaccccccgttcagcccgaccgctgcgccttatccggtaactatcgtcttgagtccaacccggtaagacacgacttatcgccactggcagcagccactggtaacaggattagcagagcgaggtatgtaggcggtgctacagagttcttgaagtggtggcctaactacggctacactagaaggacagtatttggtatctgcgctctgctgaagccagttaccttcggaaaaagagttggtagctcttgatccggcaaacaaaccaccgctggtagcggtggtttttttgtttgcaagcagcagattacgcgcagaaaaaaaggatctcaagaagatcctttgatcttttctacggggtctgacgctcagtggaacgaaaactcacgttaagggattttggtcatgagattatcaaaaaggatcttcacctagatccttttaaattaaaaatgaagttttaaatcaatctaaagtatatatgagtaaacttggtctgacagttaccaatgcttaatcagtgaggcacctatctcagcgatctgtctatttcgttcatccatagttgcctgactccccgtcgtgtagataactacgatacgggagggcttaccatctggccccagtgctgcaatgataccgcgagacccacgctcaccggctccagatttatcagcaataaaccagccagccggaagggccgagcgcagaagtggtcctgcaactttatccgcctccatccagtctattaattgttgccgggaagctagagtaagtagttcgccagttaatagtttgcgcaacgttgttgccattgctacaggcatcgtggtgtcacgctcgtcgtttggtatggcttcattcagctccggttcccaacgatcaaggcgagttacatgatcccccatgttgtgcaaaaaagcggttagctccttcggtcctccgatcgttgtcagaagtaagttggccgcagtgttatcactcatggttatggcagcactgcataattctcttactgtcatgccatccgtaagatgcttttctgtgactggtgagtactcaaccaagtcattctgagaatagtgtatgcggcgaccgagttgctcttgcccggcgtcaatacgggataataccgcgccacatagcagaactttaaaagtgctcatcattggaaaacgttcttcggggcgaaaactctcaaggatcttaccgctgttgagatccagttcgatgtaacccactcgtgcacccaactgatcttcagcatcttttactttcaccagcgtttctgggtgagcaaaaacaggaaggcaaaatgccgcaaaaaagggaataagggcgacacggaaatgttgaatactcatactcttcctttttcaatattattgaagcatttatcagggttattgtctcatgagcggatacatatttgaatgtatttagaaaaataaacaaataggggttccgcgcacatttccccgaaaagtgccacctg

SEQ ID NO: 6 - DNA, 4724 bp, synthetic construct
  source 1..4724: mol_type = other DNA
gtcgacattgattattgactagttattaatagtaatcaattacggggtcattagttcatagcccatatatggagttccgcgttacataacttacggtaaatggcccgcctggctgaccgcccaacgacccccgcccattgacgtcaataatgacgtatgttcccatagtaacgccaatagggactttccattgacgtcaatgggtggactatttacggtaaactgcccacttggcagtacatcaagtgtatcatatgccaagtacgccccctattgacgtcaatgacggtaaatggcccgcctggcattatgcccagtacatgaccttatgggactttcctacttggcagtacatctacgtattagtcatcgctattaccatgggtcgaggtgagccccacgttctgcttcactctccccatctcccccccctccccacccccaattttgtatttatttattttttaattattttgtgcagcgatgggggcggggggggggggggcgcgcgccaggcggggcggggcggggcgaggggcggggcggggcgaggcggagaggtgcggcggcagccaatcagagcggcgcgctccgaaagtttccttttatggcgaggcggcggcggcggcggccctataaaaagcgaagcgcgcggcgggcgggagtcgctgcgttgccttcgccccgtgccccgctccgcgccgcctcgcgccgcccgccccggctctgactgaccgcgttactcccacaggtgagcgggcgggacggcccttctcctccgggctgtaattagcgcttggtttaatgacggctcgtttcttttctgtggctgcgtgaaagccttaaagggctccgggagggccctttgtgcgggggggagcggctcggggggtgcgtgcgtgtgtgtgtgcgtggggagcgccgcgtgcggcccgcgctgcccggcggctgtgagcgctgcgggcgcggcgcggggctttgtgcgctccgcgtgtgcgcgaggggagcgcggccgggggcggtgccccgcggtgcgggggggctgcgaggggaacaaaggctgcgtgcggggtgtgtgcgtgggggggtgagcagggggtgtgggcgcggcggtcgggctgtaacccccccctgcacccccctccccgagttgctgagcacggcccggcttcgggtgcggggctccgtgcggggcgtggcgcggggctcgccgtgccgggcggggggtggcggcaggtgggggtgccgggcggggcggggccgcctcgggccggggagggctcgggggaggggcgcggcggccccggagcgccggcggctgtcgaggcgcggcgagccgcagccattgccttttatggtaatcgtgcgagagggcgcagggacttcctttgtcccaaatctgtgcggagccgaaatctgggaggcgccgccgcaccccctctagcgggcgcggggcgaagcggtgcggcgccggcaggaaggaaatgggcggggagggccttcgtgcgtcgccgcgccgccgtccccttctccctctccagcctcggggctgtccgcggggggacggctgccttcgggggggacggggcagggcggggttcggcttctggcgtgtgaccggcggctctagagcctctgctaaccatgttcatgccttcttctttttcctacagctcctgggcaacgtgctggttattgtgctgtctcatcattttggcaaagaattcggcggccgcgctagcagatctttttccctctgccaaaaattatggggacatcatgaagccccttgagcatctgacttctggctaataaaggaaatttattttcattgcaatagtgtgttggaattttttgtgtctctcactcggaaggacatatgggagggcaaatcatttaaaacatcagaatgagtatttggtttagagtttggcaacatatgcccatatgctggctgccatgaacaaaggttggctataaagaggtcatcagtatatgaaacagccccctgctgtccattccttattccatagaaaagccttgacttgaggttagattttttttatattttgttttgtgttatttttttctttaacatccctaaaattttccttacatgttttactagccagatttttcctcctctcctgactactcccagtcatagctgtccctcttctcttatggagatccctcgacctgcagcccaagcttggcgtaatcatggtcatagctgtttcctgtgtgaaattgttatccgctcacaattccacacaacatacgagccggaagcataaagtgtaaagcctggggtgcctaatgagtgagctaactcacattaattgcgttgcgctcactgcccgctttccagtcgggaaacctgtcgtgccagcggatccgcatctcaattagtcagcaaccatagtcccgcccctaactccgcccatcccgcccctaactccgcccagttccgcccattctccgccccatggctgactaattttttttatttatgcagaggccgaggccgcctcggcctctgagctattccagaagtagtgaggaggcttttttggaggcctaggcttttgcaaaaagctaacttgtttattgcagcttataatggttacaaataaagcaatagcatcacaaatttcacaaataaagcatttttttcactgcattctagttgtggtttgtccaaactcatcaatgtatcttatcatgtctggatccgctgcattaatgaatcggccaacgcgcggggagaggcggtttgcgtattgggcgctcttccgcttcctcgctcactgactcgctgcgctcggtcgttcggctgcggcgagcggtatcagctcactcaaaggcggtaatacggttatccacagaatcaggggataacgcaggaaagaacatgtgagcaaaaggccagcaaaaggccaggaaccgtaaaaaggccgcgttgctggcgtttttccataggctccgcccccctgacgagcatcacaaaaatcgacgctcaagtcagaggtggcgaaacccgacaggactataaagataccaggcgtttccccctggaagctccctcgtgcgctctcctgttccgaccctgccgcttaccggatacctgtccgcctttctcccttcgggaagcgtggcgctttctcaatgctcacgctgtaggtatctcagttcggtgtaggtcgttcgctccaagctgggctgtgtgcacgaaccccccgttcagcccgaccgctgcgccttatccggtaactatcgtcttgagtccaacccggtaagacacgacttatcgccactggcagcagccactggtaacaggattagcagagcgaggtatgtaggcggtgctacagagttcttgaagtggtggcctaactacggctacactagaaggacagtatttggtatctgcgctctgctgaagccagttaccttcggaaaaagagttggtagctcttgatccggcaaacaaaccaccgctggtagcggtggtttttttgtttgcaagcagcagattacgcgcagaaaaaaaggatctcaagaagatcctttgatcttttctacggggtctgacgctcagtggaacgaaaactcacgttaagggattttggtcatgagattatcaaaaaggatcttcacctagatccttttaaattaaaaatgaagttttaaatcaatctaaagtatatatgagtaaacttggtctgacagttaccaatgcttaatcagtgaggcacctatctcagcgatctgtctatttcgttcatccatagttgcctgactccccgtcgtgtagataactacgatacgggagggcttaccatctggccccagtgctgcaatgataccgcgagacccacgctcaccggctccagatttatcagcaataaaccagccagccggaagggccgagcgcagaagtggtcctgcaactttatccgcctccatccagtctattaattgttgccgggaagctagagtaagtagttcgccagttaatagtttgcgcaacgttgttgccattgctacaggcatcgtggtgtcacgctcgtcgtttggtatggcttcattcagctccggttcccaacgatcaaggcgagttacatgatcccccatgttgtgcaaaaaagcggttagctccttcggtcctccgatcgttgtcagaagtaagttggccgcagtgttatcactcatggttatggcagcactgcataattctcttactgtcatgccatccgtaagatgcttttctgtgactggtgagtactcaaccaagtcattctgagaatagtgtatgcggcgaccgagttgctcttgcccggcgtcaatacgggataataccgcgccacatagcagaactttaaaagtgctcatcattggaaaacgttcttcggggcgaaaactctcaaggatcttaccgctgttgagatccagttcgatgtaacccactcgtgcacccaactgatcttcagcatcttttactttcaccagcgtttctgggtgagcaaaaacaggaaggcaaaatgccgcaaaaaagggaataagggcgacacggaaatgttgaatactcatactcttcctttttcaatattattgaagcatttatcagggttattgtctcatgagcggatacatatttgaatgtatttagaaaaataaacaaataggggttccgcgcacatttccccgaaaagtgccacctg

SEQ ID NO: 7 - DNA, 2967 bp, synthetic construct
  source 1..2967: mol_type = other DNA
atgagtctggccattccagttatgtgcctgctggcaaataccacgttcccctgctcccagcccccttgcacaccctgctgctacgaaaaagagccggagaaaaccttgcgcatgcttgaagacaatgtcatgagccccgggtactatcagctgctacaagcatccttaacatgttctccccgacgccagcggcgcagtattaaggaccacttcaatgtctataaagccacaagaccgtacctagctcactgtcccgactgtggagaagggcactcgtgccatagtcccgtagcgctagaacgcatcagaaacgaagcgacagacgggacgttgaaaatccaggtttccttgcaaatcggaataaagacggatgatagccatgattggaccaagctgcgttatatggacaatcacatgccagcagacgcagagcgggccgggctatttgtaagaacgtcagcaccgtgcacgattactggaacaatgggacacttcattctggcccgatgtccgaaaggagaaactctgacggtagggttcactgacggtaggaagatcagtcactcatgtacgcacccatttcaccatgaccctcctgtgataggccgggaaaaattccattcccgaccgcagcacggtagggaactaccttgcagcacgtacgcgcagagcaccgctgcaactgccgaggagatagaggtacatatgcccccagacaccccagatcgcacattaatgtcacaacagtccggcaatgtaaagatcacagtcaatagtcagacggtgcggtacaagtgcaattgtggtgactcaagtgaaggattaaccactacagataaagtgattaataactgcaaggttgatcaatgccatgccgcggtcaccaatcacaaaaaatggcagtataattcccctctggtcccgcgtaatgctgaattcggggaccggaaaggaaaagttcacattccatttcctctggcaaatgtgacatgcagggtgcctaaagcaagaaaccccaccgtgacgtacggaaaaaaccaagtcatcatgttgctgtatcctgaccacccaacgctcctgtcctacaggaatatgggagaagaaccaaactatcaagaagagtgggtgacgcataagaaggagatcaggttaaccgtgccgactgaagggctcgaggtcacgtggggtaacaatgagccgtacaagtattggccgcagttatccacaaacggtacagcccacggccacccgcatgagataattctgtattattatgagctgtacccaactatgactgtggtagttttgtcagtggcctcgttcatactcctgtcgatggtgggtgtggcagtggggatgtgcatgtgtgcacgacgcagatgcattacaccgtacgaactgacaccaggagctaccgtccctttcctgcttagcctaatatgctgcattagaacagctaaagcggccacataccaggaggccgcggtatacctgtggaacgagcagcagcctttattttggctgcaagcccttattccgctggcagccctgattgtcctatgtaactgtctgagactcttaccatgctgttgtaaaatgttgacttttttagccgtactgagcgtcggtgcccacactgtgagtgcgtacgaacacgtaacagtgatcccgaacacggtgggagtaccgtataagactctagtcaacagaccgggctacagccccatggtattggagatggagcttctgtctgtcaccttggaaccaacgctatcgcttgattacatcacgtgcgagtataaaaccgttatcccgtctccgtacgtgaaatgctgcggtacagcagagtgtaaggacaagagcctacctgattacagctgtaaggtcttcaccggcgtctacccattcatgtggggcggcgcctactgcttctgcgacaccgaaaatacgcaattgagcgaagcacatgtggagaagtccgaatcatgcaaaacagaatttgcatcagcatacagggctcataccgcatccgcgtcagctaagctccgcgtcctttaccaaggaaataatatcactgtagctgcttatgcaaacggcgaccatgccgtcacagttaaggacgctaaattcatagtggggccaatgtcttcagcctggacacctttcgacaataaaatcgtggtgtacaaaggcgacgtctacaacatggactacccgcccttcggcgcaggaagaccaggacaatttggcgacatccaaagtcgcacgcctgagagcgaagacgtctatgctaatacacaactggtactgcagagaccgtccgcgggtacggtgcacgtgccgtactctcaggcaccatctggcttcaagtattggctaaaagaacgaggggcgtcgctgcagcacacagcaccatttggctgtcaaatagcaacaaacccggtaagagcgatgaactgcgccgtagggaacatgcctatctccatcgacataccggacgcggcctttaccagggtcgtcgacgcgccatctttaacggacatgtcgtgtgaggtatcagcctgcacccattcctcagactttgggggcgtagccatcattaaatatgcagccagtaagaaaggcaagtgtgcagtgcactcgatgactaacgccgtcactattcgggaagctgaaatagaagtagaagggaactctcagttgcaaatctctttttcgacggccctagccagcgccgaatttcgcgtacaagtctgttctacacaagtacactgtgcagccgagtgccatccaccgaaagaccatatagtcaattacccggcgtcacacaccaccctcggggtccaagacatttccgctacggcgatgtcatgggtgcagaagatcacgggaggtgtgggactggttgtcgctgttgcagcactgatcctaatcgtggtgctatgcgtgtcgtttagcaggcactaa

SEQ ID NO: 8 - DNA, 2946 bp, synthetic construct
  source 1..2946: mol_type = other DNA
atgtcactagtgaccaccatgtgtctgctcgccaatgtgacgttcccatgtgctcaaccaccaatttgctacgacagaaaaccagcagagactttggccatgctcagcgttaacgttgacaacccgggctacgatgagctgctggaagcagctgttaagtgccccggaaggaaaaggagatccaccgaggagctgtttaatgagtataagctaacgcgcccttacatggccagatgcatcagatgtgcagttgggagctgccatagtccaatagcaatcgaggcagtaaagagcgacgggcacgacggttatgttagacttcagacttcctcgcagtatggcctggattcctccggcaacttaaagggcaggaccatgcggtatgacatgcacgggaccattaaagagataccactacatcaagtgtcactctatacatctcgcccgtgtcacattgtggatgggcacggttatttcctgcttgccaggtgcccggcaggggactccatcaccatggaatttaagaaagattccgtcagacactcctgctcggtgccgtatgaagtgaaatttaatcctgtaggcagagaactctatactcatcccccagaacacggagtagagcaagcgtgccaagtctacgcacatgatgcacagaacagaggagcttatgtcgagatgcacctcccgggctcagaagtggacagcagtttggtttccttgagcggcagttcagtcaccgtgacacctcctgatgggactagcgccctggtggaatgcgagtgtggcggcacaaagatctccgagaccatcaacaagacaaaacagttcagccagtgcacaaagaaggagcagtgcagagcatatcggctgcagaacaataagtgggtgtataattctgacaaactgcccaaagcagcgggagccaccttaaaaggaaaactgcatgtcccattcttgctggcagacggcaaatgcaccgtgcctctagcaccagaacctatgataaccttcggtttcagatcagtgtcactgaaactgcaccctaagaatcccacatatctaaccacccgccaacttgctgatgagcctcactacacgcacgagctcatatctgaaccagctgttaggaattttaccgtcaccgaaaaagggtgggagtttgtatggggaaaccacccgccgaaaaggttttgggcacaggaaacagcacccggaaatccacatgggctaccgcacgaggtgataactcattattaccacagataccctatgtccaccatcctgggtttgtcaatttgtgccgccattgcaaccgtttccgttgcagcgtctacctggctgttttgcagatctagagttgcgtgcctaactccttaccggctaacacctaacgctaggataccattttgtctggctgtgctttgctgcgcccgcactgcccgggccgagaccacctgggagtccttggatcacctatggaacaataaccaacagatgttctggattcaattgctgatccctctggccgccttgatcgtagtgactcgcctgctcaggtgcgtgtgctgtgtcgtgccttttttagtcatggccggcgccgcaggcgccggcgcctacgagcacgcgaccacgatgccgagccaagcgggaatctcgtataacactatagtcaacagagcaggctacgcaccactccctatcagcataacaccaacaaagatcaagctgatacctacagtgaacttggagtacgtcacctgccactacaaaacaggaatggattcaccagccatcaaatgctgcggatctcaggaatgcactccaacttacaggcctgatgaacagtgcaaagtcttcacaggggtttacccgttcatgtggggtggtgcatattgcttttgcgacactgagaacacccaagtcagcaaggcctacgtaatgaaatctgacgactgccttgcggatcatgctgaagcatataaagcgcacacagcctcagtgcaggcgttcctcaacatcacagtgggagaacactctattgtgactaccgtgtatgtgaatggagaaactcctgtgaatttcaatggggtcaaaataactgcaggtccgctttccacagcttggacaccctttgatcgcaaaatcgtgcagtatgccggggagatctataattatgattttcctgagtatggggcaggacaaccaggagcatttggagatatacaatccagaacagtctcaagctctgatctgtatgccaataccaacctagtgctgcagagacccaaagcaggagcgatccacgtgccatacactcaggcaccttcgggttttgagcaatggaagaaagataaagctccatcattgaaatttaccgcccctttcggatgcgaaatatatacaaaccccattcgcgccgaaaactgtgctgtagggtcaattccattagcctttgacattcccgacgccttgttcaccagggtgtcagaaacaccgacactttcagcggccgaatgcactcttaacgagtgcgtgtattcttccgactttggtgggatcgccacggtcaagtactcggccagcaagtcaggcaagtgcgcagtccatgtgccatcagggactgctaccctaaaagaagcagcagtcgagctaaccgagcaagggtcggcgactatccatttctcgaccgcatatatccacccggagttcaggctccaaatatgcacatcatatgttacgtgcaaaggtgattgtcaccccccgaaagaccattttgtgacacaccctcagtatcacgcccaaacatttacagccgcggtgtcaaaaaccgcgtggacgtggttaacatccctgctgggaggatcagccgtaattattataattggcttggtgctggctactattgtggccatgtacgtgctgaccaaccagaaacataattga

SEQ ID NO: 9 - DNA, 2039 bp, synthetic construct
  source 1..2039: mol_type = other DNA
atgggcgttacaggaatattgcagttacctcgtgatcgattcaagaggacatcattctttctttgggtaattatccttttccaaagaacattttccatcccacttggagtcatccacaatagcacattacaggttagtgatgtcgacaaactagtttgtcgtgacaaactgtcatccacaaatcaattgagatcagttggactgaatctcgaagggaatggagtggcaactgacgtgccatctgcaactaaaagatggggcttcaggtccggtgtcccaccaaaggtggtcaattatgaagctggtgaatgggctgaaaactgctacaatcttgaaatcaaaaaacctgacgggagtgagtgtctaccagcagcgccagacgggattcggggcttcccccggtgccggtatgtgcacaaagtatcaggaacgggaccgtgtgccggagactttgccttccataaagagggtgctttcttcctgtatgatcgacttgcttccacagttatctaccgaggaacgactttcgctgaaggtgtcgttgcatttctgatactgccccaagctaagaaggacttcttcagctcacaccccttgagagagccggtcaatgcaacggaggacccgtctagtggctactattctaccacaattagatatcaggctaccggttttggaaccaatgagacagagtacttgttcgaggttgacaatttgacctacgtccaacttgaatcaagattcacaccacagtttctgctccagctgaatgagacaatatatacaagtgggaaaaggagcaataccacgggaaaactaatttggaaggtcaaccccgaaattgatacaacaatcggggagtgggccttctgggaaactaaaaaaaacctcactagaaaaattcgcagtgaagagttgtctttcacagttgtatcaaacggagccaaaaacatcagtggtcagagtccggcgcgaacttcttccgacccagggaccaacacaacaactgaagaccacaaaatcatggcttcagaaaattcctctgcaatggttcaagtgcacagtcaaggaagggaagctgcagtgtcgcatctaacaacccttgccacaatctccacgagtccccaatccctcacaaccaaaccaggtccggacaacagcacccataatacacccgtgtataaacttgacatctctgaggcaactcaagttgaacaacatcaccgcagaacagacaacgacagcacagcctccgacactccctctgccacgaccgcagccggacccccaaaagcagagaacaccaacacgagcaagagcactgacttcctggaccccgccaccacaacaagtccccaaaaccacagcgagaccgctggcaacaacaacactcatcaccaagataccggagaagagagtgccagcagcgggaagctaggcttaattaccaatactattgctggagtcgcaggactgatcacaggcgggagaagaactcgaagagaagcaattgtcaatgctcaacccaaatgcaaccctaatttacattactggactactcaggatgaaggtgctgcaatcggactggcctggataccatatttcgggccagcagccgagggaatttacatagaggggctaatgcacaatcaagatggtttaatctgtgggttgagacagctggccaacgagacgactcaagctcttcaactgttcctgagagccacaactgagctacgcaccttttcaatcctcaaccgtaaggcaattgatttcttgctgcagcgatggggcggcacatgccacattctgggaccggactgctgtatcgaaccacatgattggaccaagaacataacagacaaaattgatcagattattcatgattttgttgataaaacccttccggaccagggggacaatgacaattggtggacaggatggagacaatggataccggcaggtattggagttacaggcgttataattgcagttatcgctttattctgtatatgcaaatttgtcttttagttaattaa

SEQ ID NO: 10 - DNA, 3532 bp, synthetic construct
  source 1..3532: mol_type = other DNA
atgccggcagaaaacaagaaagttagattcgaaaatactacttcagacaaagggaaaattcctagtaaagttattaagagctactacggaaccatggacattaagaaaataaatgaaggattattggacagcaaaatattaagtgctttcaacacagtaatagcattgcttggatctatcgtgatcatagtgatgaatataatgatcatccaaaattacacaagatcaacagacaatcaggccgtgatcaaagatgcgttgcagggtatccaacagcagatcaaagggcttgctgacaaaatcggcacagagatagggcccaaagtatcactgattgacacatccagtaccattactatcccagctaacattgggctgttaggttcaaagatcagccagtcgactgcaagtataaatgagaatgtgaatgaaaaatgcaaattcacactgcctcccttgaaaatccacgaatgtaacatttcttgtcctaacccactcccttttagagagtataggccacagacagaaggggtgagcaatctagtaggattacctaataatatttgcctgcaaaagacatctaatcagatattgaagccaaagctgatttcatacactttacccgtagtcggtcaaagtggtacctgtatcacagacccattgctggctatggacgagggctattttgcatatagccacctggaaagaatcggatcatgttcaagaggggtctccaaacaaagaataataggagttggagaggtactagacagaggtgatgaagttccttctttatttatgaccaatgtctggaccccaccaaatccaaacaccgtttaccactgtagtgctgtatacaacaatgaattctattatgtactttgtgcagtgtcaactgttggagaccctattctgaatagcacctactggtccggatctctaatgatgacccgtctagctgtgaaacccaagagtaatggtgggggttacaatcaacatcaacttgccctacgaagtatcgagaaagggaggtatgataaagttatgccgtatggaccttcaggcatcaaacagggtgacaccctgtattttcctgctgtaggatttttggtcaggacagagtttaaatacaatgattcaaattgtcccatcacgaagtgtcaatacagtaaacctgaaaattgcaggctatctatggggattagaccaaacagccattatatccttcgatctggactattaaaatacaatctatcagatggggagaaccccaaagttgtattcattgaaatatctgatcaaagattatctattggatctcctagcaaaatctatgattctttgggtcaacctgttttctaccaagcgtcattttcatgggatactatgattaaatttggagatgttctaacagtcaaccctctggttgtcaattggcgtaataacacggtaatatcaagacccgggcaatcacaatgccctagattcaatacatgtccagagatctgctgggaaggagtttataatgatgcattcctaattgacagaatcaattggataagcgcgggtgtattccttgacagcaatcagaccgcagaaaatcctgtttttactgtattcaaagataatgaaatactttatagggcacaactggcttctgaggacaccaatgcacaaaaaacaataactaattgttttctcttgaagaataagatttggtgcatatcattggttgagatatatgacacaggagacaatgtcataagacccaaactattcgcggttaagataccagagcaatgtacataattaattaatacctgagaggggcccctataactctctacggctaacctgaatggactacgacatagtctagtccgccaagaccatggtagttatacttgacaagagatgttattgtaatcttttaatattgattttgatgatctcggagtgtagtgttgggattctacattatgagaaattgagtaaaattggacttgtcaaaggagtaacaagaaaatacaagattaaaagcaatcctctcacaaaagacattgttataaaaatgattccgaatgtgtcgaacatgtctcagtgcacagggagtgtcatggaaaattataaaacacgattaaacggtatcttaacacctataaagggagcgttagagatctacaaaaacaacactcatgaccttgtcggtgatgtgagattagccggagttataatggcaggagttgctattgggattgcaaccgcagctcaaatcactgcaggtgtagcactatatgaggcaatgaagaatgctgacaacatcaacaaactcaaaagcagcattgaatcaactaatgaagctgtcgttaaacttcaagagactgcagaaaagacagtctatgtgctgactgctctacaggattacattaatactaatttagtaccgacaattgacaagataagctgcaaacagacagaactctcactagatctggcattatcaaagtacctctctgatttgctttttgtatttggccccaaccttcaagacccagtttctaattcaatgactatacaggctatatctcaggcattcggtggaaattatgaaacactgctaagaacattgggttacgctacagaagactttgatgatcttctagaaagtgacagcataacaggtcaaatcatctatgttgatctaagtagctactatataattgtcagggtttattttcctattctgactgaaattcaacaggcctatatccaagagttgttaccagtgagcttcaacaatgataattcagaatggatcagtattgtcccaaatttcatattggtaaggaatacattaatatcaaatatagagattggattttgcctaattacaaagaggagcgtgatctgcaaccaagattatgccacacctatgaccaacaacatgagagaatgtttaacgggatcgactgagaagtgtcctcgagagctggttgtttcatcacatgttcccagatttgcactatctaacggggttctgtttgccaattgcataagtgttacatgtcagtgtcaaacaacaggcagggcaatctcacaatcaggagaacaaactctgctgatgattgacaacaccacctgtcctacagccgtactcggtaatgtgattatcagcttagggaaatatctggggtcagtaaattataattctgaaggcattgctatcggtcctccagtctttacagataaagttgatatatcaagtcagatatccagcatgaatcagtccttacaacagtctaaggactatatcaaagaggctcaacgactccttgatactgttaatccatcattaataagcatgttgtctatgatcatactgtatgtattatcgatcgcatcgttgtgtatagggttgattacatttatcagttttatcattgttgagaaaaagagaaacacctacagcagattagaggataggagagtcagacctacaagcagtggggatctctactacattgggacatag

SEQ ID NO: 11 - DNA, 1476 bp, synthetic construct
  source 1..1476: mol_type = other DNA
atgggacaaatagtgacattcttccaggaagtgcctcatgtaatagaagaggtgatgaacattgttctcattgcactgtctgtactagcagtgctgaaaggtctgtacaattttgcaacgtgtggccttgttggtttggtcactttcctcctgttgtgtggtaggtcttgcacaaccagtctttataaaggggtttatgagcttcagactctggaactaaacatggagacactcaatatgaccatgcctctctcctgcacaaagaacaacagtcatcattatataatggtgggcaatgagacaggactagaactgaccttgaccaacacgagcattattaatcacaaattttgcaatctgtctgatgcccacaaaaagaacctctatgaccacgctcttatgagcataatctcaactttccacttgtccatccccaacttcaatcagtatgaggcaatgagctgcgattttaatgggggaaagattagtgtgcagtacaacctgagtcacagctatgctggggatgcagccaaccattgtggtactgttgcaaatggtgtgttacagacttttatgaggatggcttggggtgggagctacattgctcttgactcaggccgtggcaactgggactgtattatgactagttatcaatatctgataatccaaaatacaacctgggaagatcactgccaattctcgagaccatctcccatcggttatctcgggctcctctcacaaaggactagagatatttatattagtagaagattgctaggcacattcacatggacactgtcagattctgaaggtaaagacacaccagggggatattgtctgaccaggtggatgctaattgaggctgaactaaaatgcttcgggaacacagctgtggcaaaatgtaatgagaagcatgatgaggaattttgtgacatgctgaggctgtttgacttcaacaaacaagccattcaaaggttgaaagctgaagcacaaatgagcattcagttgatcaacaaagcagtaaatgctttgataaatgaccaacttataatgaagaaccatctacgggacatcatgggaattccatactgtaattacagcaagtattggtacctcaaccacacaactactgggagaacatcactgcccaaatgttggcttgtatcaaatggttcatacttgaacgagacccacttttctgatgatattgaacaacaagctgacaatatgatcactgagatgttacagaaggagtatatggagaggcaggggaagacaccattgggtctagttgacctctttgtgttcagtacaagtttctatcttattagcatcttccttcacctagtcaaaataccaactcataggcatattgtaggcaagtcgtgtcccaaacctcacagattgaatcatatgggcatttgttcctgtggactctacaaacagcctggtgtgcctgtgaaatggaagagatga

SEQ ID NO: 12 - DNA, 1572 bp, synthetic construct
  source 1..1572: mol_type = other DNA
atggttcctcaggctctcctgtttgtaccccttctggtttttccattgtgttttgggaaattccctatttacacgataccagacaagcttggtccctggagtccgattgacatacatcacctcagctgcccaaacaatttggtagtggaggacgaaggatgcaccaacctgtcagggttctcctacatggaacttaaagttggatacatcttagccataaaagtgaacgggttcacttgcacaggcgttgtgacggaggctgaaacctacactaacttcgttggttatgtcacaaccacgttcaaaagaaagcatttccgcccaacaccagatgcatgtagagccgcgtacaactggaagatggccggtgaccccagatatgaagagtctctacacaatccgtaccctgactaccgctggcttcgaactgtaaaaaccaccaaggagtctctcgttatcatatctccaagtgtggcagatttggacccatatgacagatcccttcactcgagggtcttccctagcgggaagtgctcaggagtagcggtgtcttctacctactgctccactaaccacgattacaccatttggatgcccgagaatccgagactagggatgtcttgtgacatttttacctccagtagagggaagagagcatccaaagggagtgagacttgcggctttgtagatgaaagaggcctatataagtctttaaaaggagcatgcaaactcaagttatgtggagttctaggacttagacttatggatggaacatgggtctcgatgcaaacatcaaatgaaaccaaatggtgccctcccgataagttggtgaacctgcacgactttcgctcagacgaaattgagcaccttgttgtagaggagttggtcaggaagagagaggagtgtctggatgcactagagtccatcatgacaaccaagtcagtgagtttcagacgtctcagtcatttaagaaaacttgtccctgggtttggaaaagcatataccatattcaacaagaccttgatggaagccgatgctcactacaagtcagtcgaaacttggaatgagatcctcccttcaaaagggtgtttaagagttggggggaggtgtcatcctcatgtgaacggggtgtttttcaatggtataatattaggacctgacggcaatgtcttaatcccagagatgcaatcatccctcctccagcaacatatggagttgttggaatcctcggttatcccccttgtgcaccccctggcagacccgtctaccgttttcaaggacggtgacgaggctgaggattttgttgaagttcaccttcccgatgtgcacaatcaggtctcaggagttgacttgggtctcccgaactgggggaagtatgtattactgagtgcaggggccctgactgccttgatgttgataattttcctgatgacatgttgtagaagagtcaatcgatcagaacctacgcaacacaatctcagagggacagggagggaggtgtcagtcactccccaaagcgggaagatcatatcttcatgggaatcacacaagagtgggggtgagaccagactg

SEQ ID NO: 13 - DNA, 1350 bp, synthetic construct
  source 1..1350: mol_type = other DNA
atgaatccaaatcagaagatagtgaccattggatcaatctgtatggtaagtgggataattagcttgatgttacagattgggaacataatctcaatatgggtcagtcattcaattcaaacagggaatcaacaccaaactgaaccaatcagaaatactaatttcctcactgagaacactgtagcttcagtaacattagctggcaattcatctctttgccccatcaaaggatgggctgtacacagtaaagacaacagtataaggattgggtccaagggggatgtgtttgtaattagagagccgttcatatcatgctcccatctggaatgcagaaccttctttttgactcagggagctttactgaatgacaagcactccaacgggactttcaaagataggagccctcatagaacgctaatgagttgccctataggtgaggctccctctccatataactcgaggtttgagtctgttgcttggtcggcaagtgcttgccatgatggcaccagttggttgataattggaatttctggtccagacaatggggctgtggcggtattgaaatacaatggcataataacagacactatcaagagttggaggaataacatactgaggacccaagagtctgaatgtgcatgtatgaatggctcttgctttactgttatgacagatggaccaagtaatgggcaggcatcatataagattttcaaaatagaaaaagggaaagtagttaagtcagtcgaattgaatgcccccaattatcactatgaggaatgctcctgttatcctgaggctggcgaaatcatatgtgtgtgcagggataattggcatggctcaaacaggccatgggtatctttcaatcagaatttggagtatcaaataggatatatttgcagtggagttttcggtgacaatccacggccgaatgacggtacagggagttgtggaccagtgtcctctaacggggcatatggggtaaaagggttctcatttaaatatggcaatggtgtctggatcgggaggaccaaaagcactcattccaggagcggctttgaaatgatttgggatccaaacgggtggactggaacggacagtgagttctcgatgaaacaagatatagtagcaataactgattggtcaggatatagcgggagttttgtccagcacccagaactgacaggattggattgcatgagaccttgcttctgggttgagttaatcagagggcggcccaaagagagcacaatttggactagtgggagcagcatatctttttgtggtgtaaatagtgacactgtgagttggtcttggccagacggtgctgagttgccattcaccattgacaagtag

SEQ ID NO: 14 - DNA, 1725 bp, synthetic construct
  source 1..1725: mol_type = other DNA
atggagttgctaatcctcaaagcaaatgcaattaccacaatcctcactgcagtcacattttgttttgcttctggtcaaaacatcactgaagaattttatcaatcaacatgcagtgcagttagcaaaggctatcttagtgctctgagaactggttggtataccagtgttataactatagaattaagtaatatcaagaaaaataagtgtaatggaacagatgctaaggtaaaattgataaaacaagaattagataaatataaaaatgctgtaacagaattgcagttgctcatgcaaagcacacaagcaacaaacaatcgagccagaagagaactaccaaggtttatgaattatacactcaacaatgccaaaaaaaccaatgtaacattaagcaagaaaaggaaaagaagatttcttggttttttgttaggtgttggatctgcaatcgccagtggcgttgctgtatctaaggtcctgcacctagaaggggaagtgaacaagatcaaaagtgctctactatccacaaacaaggctgtagtcagcttatcaaatggagttagtgttttaaccagcaaagtgttagacctcaaaaactatatagataaacaattgttacctattgtgaacaagcaaagctgcagcatatcaaatatagaaactgtgatagagttccaacaaaagaacaacagactactagagattaccagggaatttagtgttaatgcaggcgtaactacacctgtaagcacttacatgttaactaatagtgaattattgtcattaatcaatgatatgcctataacaaatgatcagaaaaagttaatgtccaacaatgttcaaatagttagacagcaaagttactctatcatgtccataataaaagaggaagtcttagcatatgtagtacaattaccactatatggtgttatagatacaccctgttggaaactacacacatcccctctatgtacaaccaacacaaaagaagggtccaacatctgtttaacaagaactgacagaggatggtactgtgacaatgcaggatcagtatctttcttcccacaagctgaaacatgtaaagttcaatcaaatcgagtattttgtgacacaatgaacagtttaacattaccaagtgaagtaaatctctgcaatgttgacatattcaaccccaaatatgattgtaaaattatgacttcaaaaacagatgtaagcagctccgttatcacatctctaggagccattgtgtcatgctatggcaaaactaaatgtacagcatccaataaaaatcgtggaatcataaagacattttctaacgggtgcgattatgtatcaaataaaggggtggacactgtgtctgtaggtaacacattatattatgtaaataagcaagaaggtaaaagtctctatgtaaaaggtgaaccaataataaatttctatgacccattagtattcccctctgatgaatttgatgcatcaatatctcaagtcaacgagaagattaaccagagcctagcatttattcgtaaatccgatgaattattacataatgtaaatgctggtaaatccaccacaaatatcatgataactactataattatagtgattatagtaatattgttatcattaattgctgttggactgctcttatactgtaaggccagaagcacaccagtcacactaagcaaagatcaactgagtggtataaataatattgcatttagtaactaa

SEQ ID NO: 15 - DNA, 2415 bp, synthetic construct
  source 1..2415: mol_type = other DNA
atgtcaagctcttcctggctccttctcagccttgttgctgtaactgctgctcagtccaccattgaggaacaggccaagacatttttggacaagtttaaccacgaagccgaagacctgttctatcaaagttcacttgcttcttggaattataacaccaatattactgaagagaatgtccaaaacatgaataatgctggggacaaatggtctgcctttttaaaggaacagtccacacttgcccaaatgtatccactacaagaaattcagaatctcacagtcaagcttcagctgcaggctcttcagcaaaatgggtcttcagtgctctcagaagacaagagcaaacggttgaacacaattctaaatacaatgagcaccatctacagtactggaaaagtttgtaacccagataatccacaagaatgcttattacttgaaccaggtttgaatgaaataatggcaaacagtttagactacaatgagaggctctgggcttgggaaagctggagatctgaggtcggcaagcagctgaggccattatatgaagagtatgtggtcttgaaaaatgagatggcaagagcaaatcattatgaggactatggggattattggagaggagactatgaagtaaatggggtagatggctatgactacagccgcggccagttgattgaagatgtggaacatacctttgaagagattaaaccattatatgaacatcttcatgcctatgtgagggcaaagttgatgaatgcctatccttcctatatcagtccaattggatgcctccctgctcatttgcttggtgatatgtggggtagattttggacaaatctgtactctttgacagttccctttggacagaaaccaaacatagatgttactgatgcaatggtggaccaggcctgggatgcacagagaatattcaaggaggccgagaagttctttgtatctgttggtcttcctaatatgactcaaggattctgggaaaattccatgctaacggacccaggaaatgttcagaaagcagtctgccatcccacagcttgggacctggggaagggcgacttcaggatccttatgtgcacaaaggtgacaatggacgacttcctgacagctcatcatgagatggggcatatccagtatgatatggcatatgctgcacaaccttttctgctaagaaatggagctaatgaaggattccatgaagctgttggggaaatcatgtcactttctgcagccacacctaagcatttaaaatccattggtcttctgtcacccgattttcaagaagacaatgaaacagaaataaacttcctgctcaaacaagcactcacgattgttgggactctgccatttacttacatgttagagaagtggaggtggatggtctttaaaggggaaattcccaaagaccagtggatgaaaaagtggtgggagatgaagcgagagatagttggggtggtggaacctgtgccccatgatgaaacatactgtgaccccgcatctctgttccatgtttctaatgattactcattcattcgatattacacaaggaccctttaccaattccagtttcaagaagcactttgtcaagcagctaaacatgaaggccctctgcacaaatgtgacatctcaaactctacagaagctggacagaaactgttcaatatgctgaggcttggaaaatcagaaccctggaccctagcattggaaaatgttgtaggagcaaagaacatgaatgtaaggccactgctcaactactttgagcccttatttacctggctgaaagaccagaacaagaattcttttgtgggatggagtaccgactggagtccatatgcagaccaaagcatcaaagtgaggataagcctaaaatcagctcttggagataaagcatatgaatggaacgacaatgaaatgtacctgttccgatcatctgttgcatatgctatgaggcagtactttttaaaagtaaaaaatcagatgattctttttggggaggaggatgtgcgagtggctaatttgaaaccaagaatctcctttaatttctttgtcactgcacctaaaaatgtgtctgatatcattcctagaactgaagttgaaaaggccatcaggatgtcccggagccgtatcaatgatgctttccgtctgaatgacaacagcctagagtttctggggatacagccaacacttggacctcctaaccagccccctgtttccatatggctgattgtttttggagttgtgatgggagtgatagtggttggcattgtcatcctgatcttcactgggatcagagatcggaagaagaaaaataaagcaagaagtggagaaaatccttatgcctccatcgatattagcaaaggagaaaataatccaggattccaaaacactgatgatgttcagacctccttt